European Patent Application EP 4 303 583 A2, published January 10, 2024. Title: CSF1R INHIBITORS FOR USE IN TREATING CANCER. Applicant: DECIPHERA PHARMACEUTICALS, LLC. Application EP. The sequence listing filed with the application follows.

SEQUENCE LISTING (4 sequences)

SEQ ID NO: 1 - protein, 444 aa, synthetic construct
  REGION 1..444: note = source = /note="Description of Artificial Sequence: Synthetic polypeptide"
MHHHHHHEFYKYKQKPKYQVRWKIIESYEGNSYTFIDPTQLPYNEKWEFPRNNLQFGKTLGAGAFGKVVEATAFGLGKEDAVLKVAVKMLKSTAHADEKEALMSELKIMSHLGQHENIVNLLGACTHGGPVLVITEYCCYGDLLNFLRRKAEAMLGPSLSPGQDPEGGVDYKNIHLEKKYVRRDSGFSSQGVDTYVEMRPVSTSSNDSFSEQDLDKEDGRPLELRDLLHFSSQVAQGMAFLASKNCIHRDVAARNVLLTNGHVAKIGDFGLARDIMNDSNYIVKGNARLPVKWMAPESIFDCVYTVQSDVWSYGILLWEIFSLGLNPYPGILVNSKFYKLVKDGYQMAQPAFAPKNIYSIMQACWALEPTHRPTFQQICSFLQEQAQEDRRERDYTNLPSSSRSGGSGSSSSELEEESSSEHLTCCEQGDIAQPLLQPNNYQFC

SEQ ID NO: 2 - protein, 696 aa, synthetic construct
  REGION 1..696: note = source = /note="Description of Artificial Sequence: Synthetic polypeptide"
MEHHHHHHHHEYMPMEMAPILGYWKIKGLVQPTRLLLEYLEEKYEEHLYERDEGDKWRNKKFELGLEFPNLPYYIDGDVKLTQSMAIIRYIADKHNMLGGCPKERAEISMLEGAVDIRYGVSRIAYSKDFETLKVDFLSKLPEMLKMFEDRLCHKTYLNGDHVTHPDFMLYDALDVVLYMDPMCLDAFPKLVCFKKRIEAIPQIDKYLKSSKYIWPLQGWQATFGGGDHPPKSDLVPRHNQTSLYKKAGSAAAVLEENLYFQGTYKYLQKPMYEVQWKVVEEINGNNYVYIDPTQLPYDHKWEFPRNRLSFGKTLGAGAFGKVVEATAYGLIKSDAAMTVAVKMLKPSAHLTEREALMSELKVLSYLGNHMNIVNLLGACTIGGPTLVITEYCCYGDLLNFLRRKRDSFICSKQEDHAEAALYKNLLHSKESSCSDSTNEYMDMKPGVSYVVPTKADKRRSVRIGSYIERDVTPAIMEDDELALDLEDLLSFSYQVAKGMAFLASKNCIHRDLAARNILLTHGRITKICDFGLARDIKNDSNYVVKGNARLPVKWMAPESIFNCVYTFESDVWSYGIFLWELFSLGSSPYPGMPVDSKFYKMIKEGFRMLSPEHAPAEMYDIMKTCWDADPLKRPTFKQIVQLIEKQISESTNHIYSNLANCSPNRQKPVVDHSVRINSVGSTASSSQPLLVHDDV

SEQ ID NO: 3 - protein, 792 aa, synthetic construct
  REGION 1..792: note = source = /note="Description of Artificial Sequence: Synthetic polypeptide"
MEHHHHHHHHMAPILGYWKIKGLVQPTRLLLEYLEEKYEEHLYERDEGDKWRNKKFELGLEFPNLPYYIDGDVKLTQSMAIIRYIADKHNMLGGCPKERAEISMLEGAVLDIRYGVSRIAYSKDFETLKVDFLSKLPEMLKMFEDRLCHKTYLNGDHVTHPDFMLYDALDVVLYMDPMCLDAFPKLVCFKKRIEAIPQIDKYLKSSKYIAWPLQGWQATFGGGDHPPKSDLVPRHNQTSLYKKAGFEGDRTMKQKPRYEIRWRVIESISPDGHEYIYVDPMQLPYDSRWEFPRDGLVLGRVLGSGAFGKVVEGTAYGLSRSQPVMKVAVKMLKPTARSSEKQALMSELKIMTHLGPHLNIVNLLGACTKSGPIYIITEYCFYGDLVNYLHKNRDSFLSHHPEKPKKELDIFGLNPADESTRSYVILSFENNGDYMDMKQADTTQYVPMLERKEVSKYSDIQRSLYDRPASYKKKSMLDSEVKNLLSDDNSEGLTLLDLLSFTYQVARGMEFLASKNCVHRDLAARNVLLAQGKIVKICDFGLARDIMHDSNYVSKGSTFLPVKWMAPESIFDNLYTTLSDVWSYGILLWEIFSLGGTPYPGMMVDSTFYNKIKSGYRMAKPDHATSEVYEIMVKCWNSEPEKRPSFYHLSEIVENLLPGQYKKSYEKIHLDFLKSDHPAVARMRVDSDNAYIGVTYKNEEDKLKDWEGGLDEQRLSADSGYIIPLPDIDPVPEEEDLGKRNRHSSQTSEESAIETGSSSSTFIKREDETIEDIDMMDDIGIDSSDLVEDSFL

SEQ ID NO: 4 - protein, 419 aa, synthetic construct
  REGION 1..419: note = source = /note="Description of Artificial Sequence: Synthetic polypeptide"
MHKYKKQFRYESQLQMVQVTGSSDNEYFYVDFREYEYDLKWEFPRENLEFGKVLGSGAFGKVMNATAYGISKTGVSIQVAVKMLKEKADSSEREALMSEKMMTQLGSHENIVNLLGACTLSGPIYLIFEYCCYGDLLNYLRSKREKFHRTWTEIFKEHNFSFYPTFQSHPNSSMPGSREVQIHPDSDQISGLHGNSFHSEDEIEYENQKRLEEEEDLNVLTFEDLLCFAYQVAKGMEFLEFKSCVHRDLAARNVLVTHGKVVKICDFGLARDIMSDSNYVVRGNARLPVKWMAPESLFEGIYTIKSDVWSYGILLWEIFSLGVNPYPGIPVDANFYKLIQNGFKMDQPFYATEEIYIIMQSCWAFDSRKRPSFPNLTSFLGCQLADAEEAMYQNVKGVEACQLGTDDYDIPTTHHHHHH